European Patent Application EP 4 467 641 A1, published November 27, 2024. Title: CjCAS9 mutants with relaxed PAM compatibility. Applicant: Universität Zürich. The sequence listing filed with the application follows.

SEQUENCE LISTING (53 sequences)

SEQ ID NO: 1 - protein, 984 aa, Campylobacter jejuni
MARILAFDIGISSIGWAFSENDELKDCGVRIFTKVENPKTGESLALPRRLARSARKRLARRKARLNHLKHLIANEFKLNYEDYQSFDESLAKAYKGSLISPYELRFRALNELLSKQDFARVILHIAKRRGYDDIKNSDDKEKGAILKAIKQNEEKLANYQSVGEYLYKEYFQKFKENSKEFTNVRNKKESYERCIAQSFLKDELKLIFKKQREFGFSFSKKFEEEVLSVAFYKRALKDFSHLVGNCSFFTDEKRAPKNSPLAFMFVALTRIINLLNNLKNTEGILYTKDDLNALLNEVLKNGTLTYKQTKKLLGLSDDYEFKGEKGTYFIEFKKYKEFIKALGEHNLSQDDLNEIAKDITLIKDEIKLKKALAKYDLNQNQIDSLSKLEFKDHLNISFKALKLVTPLMLEGKKYDEACNELNLKVAINEDKKDFLPAFNETYYKDEVTNPVVLRAIKEYRKVLNALLKKYGKVHKINIELAREVGKNHSQRAKIEKEQNENYKAKKDAELECEKLGLKINSKNILKLRLFKEQKEFCAYSGEKIKISDLQDEKMLEIDHIYPYSRSFDDSYMNKVLVFTKQNQEKLNQTPFEAFGNDSAKWQKIEVLAKNLPTKKQKRILDKNYKDKEQKNFKDRNLNDTRYIARLVLNYTKDYLDFLPLSDDENTKLNDTQKGSKVHVEAKSGMLTSALRHTWGFSAKDRNNHLHHAIDAVIIAYANNSIVKAFSDFKKEQESNSAELYAKKISELDYKNKRKFFEPFSGFRQKVLDKIDEIFVSKPERKKPSGALHEETFRKEEEFYQSYGGKEGVLKALELGKIRKVNGKIVKNGDMFRVDIFKHKKTNKFYAVPIYTMDFALKVLPNKAVARSKKGEIKDWILMDENYEFCFSLYKDSLILIQTKDMQEPEFVYYNAFTSSTVSLIVSKHDNKFETLSKNQKILFKNANEKEVIAKSIGIQNLKVFEKYIVSALGEVTKAEFRQREDFKK

SEQ ID NO: 2 - protein, 984 aa, synthetic construct
MARILAFDIGISSIGWAFSENDELKDCGVRIFTKVENPKTGESLALPRRLARSARKRYARRKARLNHLKHLIANEFKLNYEDYQSFDESLAKAYKGSLISPYELRFRALNELLSKQDFARVILHIAKRRGYDDIKNSDDKEKGAILKAIKQNEEKLANYQSVGEYLYKEYFQKFKENSKEFTNVRNKKESYERCIAQSFLKDELKLIFKKQREFGFSFSKKFEEEVLSVAFYKRALKDFSHLVGNCSFFTDEKRAPKNSPLAFMFVALTRIINLLNNLKNTEGILYTKDDLNALLNEVLKNGTLTYKQTKKLLGLSDDYEFKGEKGTYFIEFKKYKEFIKALGEHNLSQDDLNEIAKDITLIKDEIKLKKALAKYDLNQNQIDSLSKLEFKDHLNISFKALKLVTPLMLEGKKYDEACNELNLKVAINEDKKDFLPAFNETYYKDEVTNPVVLRAIKEYRKVLNALLKKYGKVHKINIELAREVGKNHSQRAKIEKEQNENYKAKKDAELECEKLGLKINSKNILKLRLFKEQKEFCAYSGEKIKISDLQDEKMLEIDHIYPYSRSFDDSYMNKVLVFTKQNQEKLNQTPFEAFGNDSAKWQKIEVLAKNLPTKKQKRILDKNYKDKEQKNFKDRNLNDTRYIARLVLNYTKDYLDFLPLSDDENTKLNDTQKGSKVHVEAKSGMLTSALRHTWGFSAKDRNNHLHHAIDAVIIAYANNSIVKAFSDFKKEQESNSAELYAKKISELDYKNKRKFFEPFSGFRQKVLDKIDEIFVSKPERKKPSGALHKETFRKEEEFYQSYGGKEGVLKALELGKIRKVKGKIVKNGDMFRVDIFKHKKTNKFYAVPIYTMDFALKVLPNKAVARSKKGEIKDWILMDENYEFCFSLYKDSLILIQTKKMQEPEFVYYNAFTSSTVSLIVSKHDNKFETLSKNQKILFKNANEKEVIAKGIGIQNLKVFEKYIVSALGEVTKAEFRQREDFKK

SEQ ID NO: 3 - protein, 1221 aa, synthetic construct
MKRTADGSEFESPKKKRKVSEVEFSHEYWMRHALTLAKRARDEREVPVGAVLVLNNRVIGEGWNRAIGLHDPTAHAEIMALRQGGLVMQNYRLIDATLYVTFEPCVMCAGAMIHSRIGRVVFGVRNSKRGAAGSLMNVLNYPGMNHRVEITEGILADECAALLCDFYRMPRQVFNAQKKAQSSINSGGSSGGSSGSETPGTSESATPESSGGSSGGSARILAFAIGISSIGWAFSENDELKDCGVRIFTKVENPKTGESLALPRRLARSARKRYARRKARLNHLKHLIANEFKLNYEDYQSFDESLAKAYKGSLISPYELRFRALNELLSKQDFARVILHIAKRRGYDDIKNSDDKEKGAILKAIKQNEEKLANYQSVGEYLYKEYFQKFKENSKEFTNVRNKKESYERCIAQSFLKDELKLIFKKQREFGFSFSKKFEEEVLSVAFYKRALKDFSHLVGNCSFFTDEKRAPKNSPLAFMFVALTRIINLLNNLKNTEGILYTKDDLNALLNEVLKNGTLTYKQTKKLLGLSDDYEFKGEKGTYFIEFKKYKEFIKALGEHNLSQDDLNEIAKDITLIKDEIKLKKALAKYDLNQNQIDSLSKLEFKDHLNISFKALKLVTPLMLEGKKYDEACNELNLKVAINEDKKDFLPAFNETYYKDEVTNPVVLRAIKEYRKVLNALLKKYGKVHKINIELAREVGKNHSQRAKIEKEQNENYKAKKDAELECEKLGLKINSKNILKLRLFKEQKEFCAYSGEKIKISDLQDEKMLEIDHIYPYSRSFDDSYMNKVLVFTKQNQEKLNQTPFEAFGNDSAKWQKIEVLAKNLPTKKQKRILDKNYKDKEQKNFKDRNLNDTRYIARLVLNYTKDYLDFLPLSDDENTKLNDTQKGSKVHVEAKSGMLTSALRHTWGFSAKDRNNHLHHAIDAVIIAYANNSIVKAFSDFKKEQESNSAELYAKKISELDYKNKRKFFEPFSGFRQKVLDKIDEIFVSKPERKKPSGALHKETFRKEEEFYQSYGGKEGVLKALELGKIRKVKGKIVKNGDMFRVDIFKHKKTNKFYAVPIYTMDFALKVLPNKAVARSKKGEIKDWILMDENYEFCFSLYKDSLILIQTKKMQEPEFVYYNAFTSSTVSLIVSKHDNKFETLSKNQKILFKNANEKEVIAKGIGIQNLKVFEKYIVSALGEVTKAEFRQREDFKKSGGSKRTADGSEFEPKKKRKV

SEQ ID NO: 4 - protein, 1221 aa, synthetic construct
MKRTADGSEFESPKKKRKVSEVEFSHEYWMRHALTLAKRARDEREVPVGAVLVLNNRVIGEGWNRAIGLHDPTAHAEIMALRQGGLVMQNYRLIDATLYVTFEPCVMCAGAMIHSRIGRVVFGWRQSKRGAAGSLMNVLNYPGMNHRVEITEGILADECAALLCDFYRMPRQVFNAQKKAQSSINSGGSSGGSSGSETPGTSESATPESSGGSSGGSARILAFAIGISSIGWAFSENDELKDCGVRIFTKVENPKTGESLALPRRLARSARKRYARRKARLNHLKHLIANEFKLNYEDYQSFDESLAKAYKGSLISPYELRFRALNELLSKQDFARVILHIAKRRGYDDIKNSDDKEKGAILKAIKQNEEKLANYQSVGEYLYKEYFQKFKENSKEFTNVRNKKESYERCIAQSFLKDELKLIFKKQREFGFSFSKKFEEEVLSVAFYKRALKDFSHLVGNCSFFTDEKRAPKNSPLAFMFVALTRIINLLNNLKNTEGILYTKDDLNALLNEVLKNGTLTYKQTKKLLGLSDDYEFKGEKGTYFIEFKKYKEFIKALGEHNLSQDDLNEIAKDITLIKDEIKLKKALAKYDLNQNQIDSLSKLEFKDHLNISFKALKLVTPLMLEGKKYDEACNELNLKVAINEDKKDFLPAFNETYYKDEVTNPVVLRAIKEYRKVLNALLKKYGKVHKINIELAREVGKNHSQRAKIEKEQNENYKAKKDAELECEKLGLKINSKNILKLRLFKEQKEFCAYSGEKIKISDLQDEKMLEIDHIYPYSRSFDDSYMNKVLVFTKQNQEKLNQTPFEAFGNDSAKWQKIEVLAKNLPTKKQKRILDKNYKDKEQKNFKDRNLNDTRYIARLVLNYTKDYLDFLPLSDDENTKLNDTQKGSKVHVEAKSGMLTSALRHTWGFSAKDRNNHLHHAIDAVIIAYANNSIVKAFSDFKKEQESNSAELYAKKISELDYKNKRKFFEPFSGFRQKVLDKIDEIFVSKPERKKPSGALHKETFRKEEEFYQSYGGKEGVLKALELGKIRKVKGKIVKNGDMFRVDIFKHKKTNKFYAVPIYTMDFALKVLPNKAVARSKKGEIKDWILMDENYEFCFSLYKDSLILIQTKKMQEPEFVYYNAFTSSTVSLIVSKHDNKFETLSKNQKILFKNANEKEVIAKGIGIQNLKVFEKYIVSALGEVTKAEFRQREDFKKSGGSKRTADGSEFEPKKKRKV

SEQ ID NO: 5 - protein, 1419 aa, synthetic construct
MKRTADGSEFESPKKKRKVSEVEFSHEYWMRHALTLAKRAWDEREVPVGAVLVHNNRVIGEGWNRPIGRHDPTAHAEIMALRQGGLVMQNYRLIDATLYVTLEPCVMCAGAMIHSRIGRVVFGARDAKTGAAGSLMDVLHHPGMNHRVEITEGILADECAALLSDFFRMRRQEIKAQKKAQSSTDSGGSSGGSSGSETPGTSESATPESSGGSSGGSSEVEFSHEYWMRHALTLAKRARDEREVPVGAVLVLNNRVIGEGWNRAIGLHDPTAHAEIMALRQGGLVMQNYRLIDATLYVTFEPCVMCAGAMIHSRIGRVVFGVRNAKTGAAGSLMDVLHYPGMNHRVEITEGILADECAALLCYFFRMPRQVFNAQKKAQSSTDSGGSSGGSSGSETPGTSESATPESSGGSSGGSARILAFAIGISSIGWAFSENDELKDCGVRIFTKVENPKTGESLALPRRLARSARKRYARRKARLNHLKHLIANEFKLNYEDYQSFDESLAKAYKGSLISPYELRFRALNELLSKQDFARVILHIAKRRGYDDIKNSDDKEKGAILKAIKQNEEKLANYQSVGEYLYKEYFQKFKENSKEFTNVRNKKESYERCIAQSFLKDELKLIFKKQREFGFSFSKKFEEEVLSVAFYKRALKDFSHLVGNCSFFTDEKRAPKNSPLAFMFVALTRIINLLNNLKNTEGILYTKDDLNALLNEVLKNGTLTYKQTKKLLGLSDDYEFKGEKGTYFIEFKKYKEFIKALGEHNLSQDDLNEIAKDITLIKDEIKLKKALAKYDLNQNQIDSLSKLEFKDHLNISFKALKLVTPLMLEGKKYDEACNELNLKVAINEDKKDFLPAFNETYYKDEVTNPVVLRAIKEYRKVLNALLKKYGKVHKINIELAREVGKNHSQRAKIEKEQNENYKAKKDAELECEKLGLKINSKNILKLRLFKEQKEFCAYSGEKIKISDLQDEKMLEIDHIYPYSRSFDDSYMNKVLVFTKQNQEKLNQTPFEAFGNDSAKWQKIEVLAKNLPTKKQKRILDKNYKDKEQKNFKDRNLNDTRYIARLVLNYTKDYLDFLPLSDDENTKLNDTQKGSKVHVEAKSGMLTSALRHTWGFSAKDRNNHLHHAIDAVIIAYANNSIVKAFSDFKKEQESNSAELYAKKISELDYKNKRKFFEPFSGFRQKVLDKIDEIFVSKPERKKPSGALHKETFRKEEEFYQSYGGKEGVLKALELGKIRKVKGKIVKNGDMFRVDIFKHKKTNKFYAVPIYTMDFALKVLPNKAVARSKKGEIKDWILMDENYEFCFSLYKDSLILIQTKKMQEPEFVYYNAFTSSTVSLIVSKHDNKFETLSKNQKILFKNANEKEVIAKGIGIQNLKVFEKYIVSALGEVTKAEFRQREDFKKSGGSKRTADGSEFEPKKKRKV

SEQ ID NO: 6 - protein, 1234 aa, synthetic construct
MKRTADGSEFESPKKKRKVGSARILAFAIGISSIGWAFSENDELKDCGVRIFTKVENPKTGESLALPRRLARSARKRYARRKARLNHLKHLIANEFKLNYEDYQSFDESLAKAYKGSLISPYELRFRALNELLSKQDFARVILHIAKRRGYDDIKNSDDKEKGAILKAIKQNEEKLANYQSVGEYLYKEYFQKFKENSKEFTNVRNKKESYERCIAQSFLKDELKLIFKKQREFGFSFSKKFEEEVLSVAFYKRALKDFSHLVGNCSFFTDEKRAPKNSPLAFMFVALTRIINLLNNLKNTEGILYTKDDLNALLNEVLKNGTLTYKQTKKLLGLSDDYEFKGEKGTYFIEFKKYKEFIKALGEHNLSQDDLNEIAKDITLIKDEIKLKKALAKYDLNQNQIDSLSKLEFKDHLNISFKALKLVTPLMLEGKKYDEACNELNLKVAINEDKKDFLPAFNETYYKDEVTNPVVLRAIKEYRKVLNALLKKYGKVHKINIELGGSSEVEFSHEYWMRHALTLAKRAWDEREVPVGAVLVHNNRVIGEGWNRPIGRHDPTAHAEIMALRQGGLVMQNYRLIDATLYVTLEPCVMCAGAMIHSRIGRVVFGARDAKTGAAGSLMDVLHHPGMNHRVEITEGILADECAALLSDFFRMRRQEIKAQKKAQSSTDSGGSSGGSSGSETPGTSESATPESSGGSSGGSSEVEFSHEYWMRHALTLAKRARDEREVPVGAVLVLNNRVIGEGWNRAIGLHDPTAHAEIMALRQGGLVMQNYRLIDATLYVTFEPCVMCAGAMIHSRIGRVVFGVRNAKTGAAGSLMDVLHYPGMNHRVEITEGILADECAALLCYFFRMPRQVFNAQKKAQSSTDSGGYIARLVLNYTKDYLDFLPLSDDENTKLNDTQKGSKVHVEAKSGMLTSALRHTWGFSAKDRNNHLHHAIDAVIIAYANNSIVKAFSDFKKEQESNSAELYAKKISELDYKNKRKFFEPFSGFRQKVLDKIDEIFVSKPERKKPSGALHKETFRKEEEFYQSYGGKEGVLKALELGKIRKVKGKIVKNGDMFRVDIFKHKKTNKFYAVPIYTMDFALKVLPNKAVARSKKGEIKDWILMDENYEFCFSLYKDSLILIQTKKMQEPEFVYYNAFTSSTVSLIVSKHDNKFETLSKNQKILFKNANEKEVIAKGIGIQNLKVFEKYIVSALGEVTKAEFRQREDFKKSGGSKRTADGSEFEPKKKRKV

SEQ ID NO: 7 - protein, 1234 aa, synthetic construct
MKRTADGSEFESPKKKRKVGSARILAFAIGISSIGWAFSENDELKDCGVRIFTKVENPKTGESLALPRRLARSARKRYARRKARLNHLKHLIANEFKLNYEDYQSFDESLAKAYKGSLISPYELRFRALNELLSKQDFARVILHIAKRRGYDDIKNSDDKEKGAILKAIKQNEEKLANYQSVGEYLYKEYFQKFKENSKEFTNVRNKKESYERCIAQSFLKDELKLIFKKQREFGFSFSKKFEEEVLSVAFYKRALKDFSHLVGNCSFFTDEKRAPKNSPLAFMFVALTRIINLLNNLKNTEGILYTKDDLNALLNEVLKNGTLTYKQTKKLLGLSDDYEFKGEKGTYFIEFKKYKEFIKALGEHNLSQDDLNEIAKDITLIKDEIKLKKALAKYDLNQNQIDSLSKLEFKDHLNISFKALKLVTPLMLEGKKYDEACNELNLKVAINEDKKDFLPAFNETYYKDEVTNPVVLRAIKEYRKVLNALLKKYGKVHKINIELGGSSEVEFSHEYWMRHALTLAKRAWDEREVPVGAVLVHNNRVIGEGWNRPIGRHDPTAHAEIMALRQGGLVMQNYRLIDATLYVTLEPCVMCAGAMIHSRIGRVVFGARDAKTGAAGSLMDVLHHPGMNHRVEITEGILADECAALLSDFFRMRRQEIKAQKKAQSSTDSGGSSGGSSGSETPGTSESATPESSGGSSGGSSEVEFSHEYWMRHALTLAKRARDEREVPVGAVLVLNNRVIGEGWNRAIGLHDPTAHAEIMALRQGGLVMQNYRLIDATLYVTFEPCVMCAGAMIHSRIGRVVFGVRNSKRGAAGSLMNVLNYPGMNHRVEITEGILADECAALLCDFYRMPRQVFNAQKKAQSSTNSGGYIARLVLNYTKDYLDFLPLSDDENTKLNDTQKGSKVHVEAKSGMLTSALRHTWGFSAKDRNNHLHHAIDAVIIAYANNSIVKAFSDFKKEQESNSAELYAKKISELDYKNKRKFFEPFSGFRQKVLDKIDEIFVSKPERKKPSGALHKETFRKEEEFYQSYGGKEGVLKALELGKIRKVKGKIVKNGDMFRVDIFKHKKTNKFYAVPIYTMDFALKVLPNKAVARSKKGEIKDWILMDENYEFCFSLYKDSLILIQTKKMQEPEFVYYNAFTSSTVSLIVSKHDNKFETLSKNQKILFKNANEKEVIAKGIGIQNLKVFEKYIVSALGEVTKAEFRQREDFKKSGGSKRTADGSEFEPKKKRKV

SEQ ID NO: 8 - protein, 1469 aa, synthetic construct
MKRTADGSEFESPKKKRKVSSETGPVAVDPTLRRRIEPHEFEVFFDPRELRKETCLLYEINWGGRHSIWRHTSQNTNKHVEVNFIEKFTTERYFCPNTRCSITWFLSWSPCGECSRAITEFLSRYPHVTLFIYIARLYHHADPRNRQGLRDLISSGVTIQIMTEQESGYCWRNFVNYSPSNEAHWPRYPHLWVRLYVLELYCIILGLPPCLNILRRKQPQLTFFTIALQSCHYQRLPPHILWATGLKSGGSSGGSSGSETPGTSESATPESSGGSSGGSARILAFAIGISSIGWAFSENDELKDCGVRIFTKVENPKTGESLALPRRLARSARKRYARRKARLNHLKHLIANEFKLNYEDYQSFDESLAKAYKGSLISPYELRFRALNELLSKQDFARVILHIAKRRGYDDIKNSDDKEKGAILKAIKQNEEKLANYQSVGEYLYKEYFQKFKENSKEFTNVRNKKESYERCIAQSFLKDELKLIFKKQREFGFSFSKKFEEEVLSVAFYKRALKDFSHLVGNCSFFTDEKRAPKNSPLAFMFVALTRIINLLNNLKNTEGILYTKDDLNALLNEVLKNGTLTYKQTKKLLGLSDDYEFKGEKGTYFIEFKKYKEFIKALGEHNLSQDDLNEIAKDITLIKDEIKLKKALAKYDLNQNQIDSLSKLEFKDHLNISFKALKLVTPLMLEGKKYDEACNELNLKVAINEDKKDFLPAFNETYYKDEVTNPVVLRAIKEYRKVLNALLKKYGKVHKINIELAREVGKNHSQRAKIEKEQNENYKAKKDAELECEKLGLKINSKNILKLRLFKEQKEFCAYSGEKIKISDLQDEKMLEIDHIYPYSRSFDDSYMNKVLVFTKQNQEKLNQTPFEAFGNDSAKWQKIEVLAKNLPTKKQKRILDKNYKDKEQKNFKDRNLNDTRYIARLVLNYTKDYLDFLPLSDDENTKLNDTQKGSKVHVEAKSGMLTSALRHTWGFSAKDRNNHLHHAIDAVIIAYANNSIVKAFSDFKKEQESNSAELYAKKISELDYKNKRKFFEPFSGFRQKVLDKIDEIFVSKPERKKPSGALHKETFRKEEEFYQSYGGKEGVLKALELGKIRKVKGKIVKNGDMFRVDIFKHKKTNKFYAVPIYTMDFALKVLPNKAVARSKKGEIKDWILMDENYEFCFSLYKDSLILIQTKKMQEPEFVYYNAFTSSTVSLIVSKHDNKFETLSKNQKILFKNANEKEVIAKGIGIQNLKVFEKYIVSALGEVTKAEFRQREDFKKSGGSGGSGGSTNLSDIIEKETGKQLVIQESILMLPEEVEEVIGNKPESDILVHTAYDESTDENVMLLTSDAPEYKPWALVIQDSNGENKIKMLSGGSGGSGGSTNLSDIIEKETGKQLVIQESILMLPEEVEEVIGNKPESDILVHTAYDESTDENVMLLTSDAPEYKPWALVIQDSNGENKIKMLSGGSKRTADGSEFEPKKKRKV

SEQ ID NO: 9 - protein, 1469 aa, synthetic construct
MKRTADGSEFESPKKKRKVSSETGPVAVDPTLRRRIEPHEFEVFFDPRELRKETCLLYEIKWGTSHKIWRHSSKNTTKHVEVNFIEKFTSERHFCPSTSCSITWFLSWSPCGECSKAITEFLSQHPNVTLVIYVARLYHHMDQQNRQGLRDLVNSGVTIQIMTAPEYDYCWRNFVNYPPGKEAHWPRYPPLWMKLYALELHAGILGLPPCLNILRRKQPQLTFFTIALQSCHYQRLPPHILWATGLKSGGSSGGSSGSETPGTSESATPESSGGSSGGSARILAFAIGISSIGWAFSENDELKDCGVRIFTKVENPKTGESLALPRRLARSARKRYARRKARLNHLKHLIANEFKLNYEDYQSFDESLAKAYKGSLISPYELRFRALNELLSKQDFARVILHIAKRRGYDDIKNSDDKEKGAILKAIKQNEEKLANYQSVGEYLYKEYFQKFKENSKEFTNVRNKKESYERCIAQSFLKDELKLIFKKQREFGFSFSKKFEEEVLSVAFYKRALKDFSHLVGNCSFFTDEKRAPKNSPLAFMFVALTRIINLLNNLKNTEGILYTKDDLNALLNEVLKNGTLTYKQTKKLLGLSDDYEFKGEKGTYFIEFKKYKEFIKALGEHNLSQDDLNEIAKDITLIKDEIKLKKALAKYDLNQNQIDSLSKLEFKDHLNISFKALKLVTPLMLEGKKYDEACNELNLKVAINEDKKDFLPAFNETYYKDEVTNPVVLRAIKEYRKVLNALLKKYGKVHKINIELAREVGKNHSQRAKIEKEQNENYKAKKDAELECEKLGLKINSKNILKLRLFKEQKEFCAYSGEKIKISDLQDEKMLEIDHIYPYSRSFDDSYMNKVLVFTKQNQEKLNQTPFEAFGNDSAKWQKIEVLAKNLPTKKQKRILDKNYKDKEQKNFKDRNLNDTRYIARLVLNYTKDYLDFLPLSDDENTKLNDTQKGSKVHVEAKSGMLTSALRHTWGFSAKDRNNHLHHAIDAVIIAYANNSIVKAFSDFKKEQESNSAELYAKKISELDYKNKRKFFEPFSGFRQKVLDKIDEIFVSKPERKKPSGALHKETFRKEEEFYQSYGGKEGVLKALELGKIRKVKGKIVKNGDMFRVDIFKHKKTNKFYAVPIYTMDFALKVLPNKAVARSKKGEIKDWILMDENYEFCFSLYKDSLILIQTKKMQEPEFVYYNAFTSSTVSLIVSKHDNKFETLSKNQKILFKNANEKEVIAKGIGIQNLKVFEKYIVSALGEVTKAEFRQREDFKKSGGSGGSGGSTNLSDIIEKETGKQLVIQESILMLPEEVEEVIGNKPESDILVHTAYDESTDENVMLLTSDAPEYKPWALVIQDSNGENKIKMLSGGSGGSGGSTNLSDIIEKETGKQLVIQESILMLPEEVEEVIGNKPESDILVHTAYDESTDENVMLLTSDAPEYKPWALVIQDSNGENKIKMLSGGSKRTADGSEFEPKKKRKV

SEQ ID NO: 10 - protein, 1438 aa, synthetic construct
MKRTADGSEFESPKKKRKVDSLLMNRRKFLYQFKNVRWAKGRRETYLCYVVKRRDSATSFSLDFGYLRNKNGCHVELLFLRYISDWDLDPGRCYRVTWFTSWSPCYDCARHVADFLRGNPNLSLRIFTARLYFCEDRKAEPEGLRRLHRAGVQIAIMTFKDYFYCWNTFVENHERTFKAWEGLHENSVRLSRQLRRILLPLYEVDDLRDAFRTLGLSGGSSGGSSGSETPGTSESATPESSGGSSGGSARILAFAIGISSIGWAFSENDELKDCGVRIFTKVENPKTGESLALPRRLARSARKRYARRKARLNHLKHLIANEFKLNYEDYQSFDESLAKAYKGSLISPYELRFRALNELLSKQDFARVILHIAKRRGYDDIKNSDDKEKGAILKAIKQNEEKLANYQSVGEYLYKEYFQKFKENSKEFTNVRNKKESYERCIAQSFLKDELKLIFKKQREFGFSFSKKFEEEVLSVAFYKRALKDFSHLVGNCSFFTDEKRAPKNSPLAFMFVALTRIINLLNNLKNTEGILYTKDDLNALLNEVLKNGTLTYKQTKKLLGLSDDYEFKGEKGTYFIEFKKYKEFIKALGEHNLSQDDLNEIAKDITLIKDEIKLKKALAKYDLNQNQIDSLSKLEFKDHLNISFKALKLVTPLMLEGKKYDEACNELNLKVAINEDKKDFLPAFNETYYKDEVTNPVVLRAIKEYRKVLNALLKKYGKVHKINIELAREVGKNHSQRAKIEKEQNENYKAKKDAELECEKLGLKINSKNILKLRLFKEQKEFCAYSGEKIKISDLQDEKMLEIDHIYPYSRSFDDSYMNKVLVFTKQNQEKLNQTPFEAFGNDSAKWQKIEVLAKNLPTKKQKRILDKNYKDKEQKNFKDRNLNDTRYIARLVLNYTKDYLDFLPLSDDENTKLNDTQKGSKVHVEAKSGMLTSALRHTWGFSAKDRNNHLHHAIDAVIIAYANNSIVKAFSDFKKEQESNSAELYAKKISELDYKNKRKFFEPFSGFRQKVLDKIDEIFVSKPERKKPSGALHKETFRKEEEFYQSYGGKEGVLKALELGKIRKVKGKIVKNGDMFRVDIFKHKKTNKFYAVPIYTMDFALKVLPNKAVARSKKGEIKDWILMDENYEFCFSLYKDSLILIQTKKMQEPEFVYYNAFTSSTVSLIVSKHDNKFETLSKNQKILFKNANEKEVIAKGIGIQNLKVFEKYIVSALGEVTKAEFRQREDFKKSGGSGGSGGSTNLSDIIEKETGKQLVIQESILMLPEEVEEVIGNKPESDILVHTAYDESTDENVMLLTSDAPEYKPWALVIQDSNGENKIKMLSGGSGGSGGSTNLSDIIEKETGKQLVIQESILMLPEEVEEVIGNKPESDILVHTAYDESTDENVMLLTSDAPEYKPWALVIQDSNGENKIKMLSGGSKRTADGSEFEPKKKRKV

SEQ ID NO: 11 - protein, 1422 aa, synthetic construct
MKRTADGSEFESPKKKRKVDSLLMNRREFLYQFKNVRWAKGRRETYLCYVVKRRDSATSFSLDFGYLRNKNGCHVELLFLRYISDWDLDPGRCYRVTWFISWSPCYDCARHVADFLRGNPNLSLRIFTARLYFCEDRKAEPEGLRRLHRAGVQIAIMTFKDYFYCWNTFVENHGRTFKAWEGLHENSVRLSRQLRRILLPSGGSSGGSSGSETPGTSESATPESSGGSSGGSARILAFAIGISSIGWAFSENDELKDCGVRIFTKVENPKTGESLALPRRLARSARKRYARRKARLNHLKHLIANEFKLNYEDYQSFDESLAKAYKGSLISPYELRFRALNELLSKQDFARVILHIAKRRGYDDIKNSDDKEKGAILKAIKQNEEKLANYQSVGEYLYKEYFQKFKENSKEFTNVRNKKESYERCIAQSFLKDELKLIFKKQREFGFSFSKKFEEEVLSVAFYKRALKDFSHLVGNCSFFTDEKRAPKNSPLAFMFVALTRIINLLNNLKNTEGILYTKDDLNALLNEVLKNGTLTYKQTKKLLGLSDDYEFKGEKGTYFIEFKKYKEFIKALGEHNLSQDDLNEIAKDITLIKDEIKLKKALAKYDLNQNQIDSLSKLEFKDHLNISFKALKLVTPLMLEGKKYDEACNELNLKVAINEDKKDFLPAFNETYYKDEVTNPVVLRAIKEYRKVLNALLKKYGKVHKINIELAREVGKNHSQRAKIEKEQNENYKAKKDAELECEKLGLKINSKNILKLRLFKEQKEFCAYSGEKIKISDLQDEKMLEIDHIYPYSRSFDDSYMNKVLVFTKQNQEKLNQTPFEAFGNDSAKWQKIEVLAKNLPTKKQKRILDKNYKDKEQKNFKDRNLNDTRYIARLVLNYTKDYLDFLPLSDDENTKLNDTQKGSKVHVEAKSGMLTSALRHTWGFSAKDRNNHLHHAIDAVIIAYANNSIVKAFSDFKKEQESNSAELYAKKISELDYKNKRKFFEPFSGFRQKVLDKIDEIFVSKPERKKPSGALHKETFRKEEEFYQSYGGKEGVLKALELGKIRKVKGKIVKNGDMFRVDIFKHKKTNKFYAVPIYTMDFALKVLPNKAVARSKKGEIKDWILMDENYEFCFSLYKDSLILIQTKKMQEPEFVYYNAFTSSTVSLIVSKHDNKFETLSKNQKILFKNANEKEVIAKGIGIQNLKVFEKYIVSALGEVTKAEFRQREDFKKSGGSGGSGGSTNLSDIIEKETGKQLVIQESILMLPEEVEEVIGNKPESDILVHTAYDESTDENVMLLTSDAPEYKPWALVIQDSNGENKIKMLSGGSGGSGGSTNLSDIIEKETGKQLVIQESILMLPEEVEEVIGNKPESDILVHTAYDESTDENVMLLTSDAPEYKPWALVIQDSNGENKIKMLSGGSKRTADGSEFEPKKKRKV

SEQ ID NO: 12 - protein, 1407 aa, synthetic construct
MKRTADGSEFESPKKKRKVSEVEFSHEYWMRHALTLAKRARDERKAPVGAVLVLNNRVIGEGWNRAIGLHDPTAHAEIIALRQGGLVMQNYRLIDATLYVTFEPCVMCAGAMINSRIGRVVFGVRNSKRGAAGSLMNVLNYPGMNHRVEITEGILADECAALLCDFYRMPRQVFNAQKKAQSSINSGGSSGGSSGSETPGTSESATPESSGGSSGGSARILAFAIGISSIGWAFSENDELKDCGVRIFTKVENPKTGESLALPRRLARSARKRYARRKARLNHLKHLIANEFKLNYEDYQSFDESLAKAYKGSLISPYELRFRALNELLSKQDFARVILHIAKRRGYDDIKNSDDKEKGAILKAIKQNEEKLANYQSVGEYLYKEYFQKFKENSKEFTNVRNKKESYERCIAQSFLKDELKLIFKKQREFGFSFSKKFEEEVLSVAFYKRALKDFSHLVGNCSFFTDEKRAPKNSPLAFMFVALTRIINLLNNLKNTEGILYTKDDLNALLNEVLKNGTLTYKQTKKLLGLSDDYEFKGEKGTYFIEFKKYKEFIKALGEHNLSQDDLNEIAKDITLIKDEIKLKKALAKYDLNQNQIDSLSKLEFKDHLNISFKALKLVTPLMLEGKKYDEACNELNLKVAINEDKKDFLPAFNETYYKDEVTNPVVLRAIKEYRKVLNALLKKYGKVHKINIELAREVGKNHSQRAKIEKEQNENYKAKKDAELECEKLGLKINSKNILKLRLFKEQKEFCAYSGEKIKISDLQDEKMLEIDHIYPYSRSFDDSYMNKVLVFTKQNQEKLNQTPFEAFGNDSAKWQKIEVLAKNLPTKKQKRILDKNYKDKEQKNFKDRNLNDTRYIARLVLNYTKDYLDFLPLSDDENTKLNDTQKGSKVHVEAKSGMLTSALRHTWGFSAKDRNNHLHHAIDAVIIAYANNSIVKAFSDFKKEQESNSAELYAKKISELDYKNKRKFFEPFSGFRQKVLDKIDEIFVSKPERKKPSGALHKETFRKEEEFYQSYGGKEGVLKALELGKIRKVKGKIVKNGDMFRVDIFKHKKTNKFYAVPIYTMDFALKVLPNKAVARSKKGEIKDWILMDENYEFCFSLYKDSLILIQTKKMQEPEFVYYNAFTSSTVSLIVSKHDNKFETLSKNQKILFKNANEKEVIAKGIGIQNLKVFEKYIVSALGEVTKAEFRQREDFKKSGGSGGSGGSTNLSDIIEKETGKQLVIQESILMLPEEVEEVIGNKPESDILVHTAYDESTDENVMLLTSDAPEYKPWALVIQDSNGENKIKMLSGGSGGSGGSTNLSDIIEKETGKQLVIQESILMLPEEVEEVIGNKPESDILVHTAYDESTDENVMLLTSDAPEYKPWALVIQDSNGENKIKMLSGGSKRTADGSEFEPKKKRKV

SEQ ID NO: 13 - protein, 1749 aa, synthetic construct
MKRTADGSEFESPKKKRKVGSARILAFDIGISSIGWAFSENDELKDCGVRIFTKVENPKTGESLALPRRLARSARKRYARRKARLNHLKHLIANEFKLNYEDYQSFDESLAKAYKGSLISPYELRFRALNELLSKQDFARVILHIAKRRGYDDIKNSDDKEKGAILKAIKQNEEKLANYQSVGEYLYKEYFQKFKENSKEFTNVRNKKESYERCIAQSFLKDELKLIFKKQREFGFSFSKKFEEEVLSVAFYKRALKDFSHLVGNCSFFTDEKRAPKNSPLAFMFVALTRIINLLNNLKNTEGILYTKDDLNALLNEVLKNGTLTYKQTKKLLGLSDDYEFKGEKGTYFIEFKKYKEFIKALGEHNLSQDDLNEIAKDITLIKDEIKLKKALAKYDLNQNQIDSLSKLEFKDHLNISFKALKLVTPLMLEGKKYDEACNELNLKVAINEDKKDFLPAFNETYYKDEVTNPVVLRAIKEYRKVLNALLKKYGKVHKINIELAREVGKNHSQRAKIEKEQNENYKAKKDAELECEKLGLKINSKNILKLRLFKEQKEFCAYSGEKIKISDLQDEKMLEIDAIYPYSRSFDDSYMNKVLVFTKQNQEKLNQTPFEAFGNDSAKWQKIEVLAKNLPTKKQKRILDKNYKDKEQKNFKDRNLNDTRYIARLVLNYTKDYLDFLPLSDDENTKLNDTQKGSKVHVEAKSGMLTSALRHTWGFSAKDRNNHLHHAIDAVIIAYANNSIVKAFSDFKKEQESNSAELYAKKISELDYKNKRKFFEPFSGFRQKVLDKIDEIFVSKPERKKPSGALHKETFRKEEEFYQSYGGKEGVLKALELGKIRKVKGKIVKNGDMFRVDIFKHKKTNKFYAVPIYTMDFALKVLPNKAVARSKKGEIKDWILMDENYEFCFSLYKDSLILIQTKKMQEPEFVYYNAFTSSTVSLIVSKHDNKFETLSKNQKILFKNANEKEVIAKGIGIQNLKVFEKYIVSALGEVTKAEFRQREDFKKSGGSSGGSKRTADGSEFESPKKKRKVSGGSSGGSTLNIEDEYRLHETSKEPDVSLGSTWLSDFPQAWAETGGMGLAVRQAPLIIPLKATSTPVSIKQYPMSQEARLGIKPHIQRLLDQGILVPCQSPWNTPLLPVKKPGTNDYRPVQDLREVNKRVEDIHPTVPNPYNLLSGLPPSHQWYTVLDLKDAFFCLRLHPTSQPLFAFEWRDPEMGISGQLTWTRLPQGFKNSPTLFNEALHRDLADFRIQHPDLILLQYVDDLLLAATSELDCQQGTRALLQTLGNLGYRASAKKAQICQKQVKYLGYLLKEGQRWLTEARKETVMGQPTPKTPRQLREFLGKAGFCRLFIPGFAEMAAPLYPLTKPGTLFNWGPDQQKAYQEIKQALLTAPALGLPDLTKPFELFVDEKQGYAKGVLTQKLGPWRRPVAYLSKKLDPVAAGWPPCLRMVAAIAVLTKDAGKLTMGQPLVILAPHAVEALVKQPPDRWLSNARMTHYQALLLDTDRVQFGPVVALNPATLLPLPEEGLQHNCLDILAEAHGTRPDLTDQPLPDADHTWYTDGSSLLQEGQRKAGAAVTTETEVIWAKALPAGTSAQRAELIALTQALKMAEGKKLNVYTDSRYAFATAHIHGEIYRRRGWLTSEGKEIKNKDEILALLKALFLPKRLSIIHCPGHQKGHSAEARGNRMADQAARKAAITETPDTSTLLIENSSPSGGSKRTADGSEFESPKKKRKVGSGPAAKRVKLD

SEQ ID NO: 14 - protein, 1552 aa, synthetic construct
MKRTADGSEFESPKKKRKVGSARILAFDIGISSIGWAFSENDELKDCGVRIFTKVENPKTGESLALPRRLARSARKRYARRKARLNHLKHLIANEFKLNYEDYQSFDESLAKAYKGSLISPYELRFRALNELLSKQDFARVILHIAKRRGYDDIKNSDDKEKGAILKAIKQNEEKLANYQSVGEYLYKEYFQKFKENSKEFTNVRNKKESYERCIAQSFLKDELKLIFKKQREFGFSFSKKFEEEVLSVAFYKRALKDFSHLVGNCSFFTDEKRAPKNSPLAFMFVALTRIINLLNNLKNTEGILYTKDDLNALLNEVLKNGTLTYKQTKKLLGLSDDYEFKGEKGTYFIEFKKYKEFIKALGEHNLSQDDLNEIAKDITLIKDEIKLKKALAKYDLNQNQIDSLSKLEFKDHLNISFKALKLVTPLMLEGKKYDEACNELNLKVAINEDKKDFLPAFNETYYKDEVTNPVVLRAIKEYRKVLNALLKKYGKVHKINIELAREVGKNHSQRAKIEKEQNENYKAKKDAELECEKLGLKINSKNILKLRLFKEQKEFCAYSGEKIKISDLQDEKMLEIDAIYPYSRSFDDSYMNKVLVFTKQNQEKLNQTPFEAFGNDSAKWQKIEVLAKNLPTKKQKRILDKNYKDKEQKNFKDRNLNDTRYIARLVLNYTKDYLDFLPLSDDENTKLNDTQKGSKVHVEAKSGMLTSALRHTWGFSAKDRNNHLHHAIDAVIIAYANNSIVKAFSDFKKEQESNSAELYAKKISELDYKNKRKFFEPFSGFRQKVLDKIDEIFVSKPERKKPSGALHKETFRKEEEFYQSYGGKEGVLKALELGKIRKVKGKIVKNGDMFRVDIFKHKKTNKFYAVPIYTMDFALKVLPNKAVARSKKGEIKDWILMDENYEFCFSLYKDSLILIQTKKMQEPEFVYYNAFTSSTVSLIVSKHDNKFETLSKNQKILFKNANEKEVIAKGIGIQNLKVFEKYIVSALGEVTKAEFRQREDFKKSGGSSGGSKRTADGSEFESPKKKRKVSGGSSGGSTLNIEDEYRLHETSKEPDVSLGSTWLSDFPQAWAETGGMGLAVRQAPLIIPLKATSTPVSIKQYPMSQEARLGIKPHIQRLLDQGILVPCQSPWNTPLLPVKKPGTNDYRPVQDLREVNKRVEDIHPTVPNPYNLLSGLPPSHQWYTVLDLKDAFFCLRLHPTSQPLFAFEWRDPEMGISGQLTWTRLPQGFKNSPTLFNEALHRDLADFRIQHPDLILLQYVDDLLLAATSELDCQQGTRALLQTLGNLGYRASAKKAQICQKQVKYLGYLLKEGQRWLTEARKETVMGQPTPKTPRQLREFLGKAGFCRLFIPGFAEMAAPLYPLTKPGTLFNWGPDQQKAYQEIKQALLTAPALGLPDLTKPFELFVDEKQGYAKGVLTQKLGPWRRPVAYLSKKLDPVAAGWPPCLRMVAAIAVLTKDAGKLTMGQPLVILAPHAVEALVKQPPDRWLSNARMTHYQALLLDTDRVQFGPVVALNPSGGSKRTADGSEFESPKKKRKVGSGPAAKRVKLD

SEQ ID NO: 15 - DNA, 4987 bp, synthetic construct
  source 1..4987: mol_type = other DNA
ctgcgcgctcgctcgctcactgaggccgcccgggcaaagcccgggcgtcgggcgacctttggtcgcccggcctcagtgagcgagcgagcgcgcagagagggagtggccaactccatcactaggggttcctaccggcgcgccgggggaggctgctggtgaatattaaccaaggtcaccccagttatcggaggagcaaacaggggctaagtccacacgcgtggtaccgtctgtctgcacatttcgtagagcgagtgttccgatactctaatctccctaggcaaggttcatatttgtgtaggttacttattctccttttgttgactaagtcaataatcagaatcagcaggtttggagtcagcttggcagggatcagcagcctgggttggaaggagggggtataaaagccccttcaccaggagaagccgtcacacagatccacaagctcctggggtaagtatcaaggttacaagacaggtttaaggagaccaatagaaactgggcttgtcgagacagagaagactcttgcgtttctgataggcacctattggtcttactgacatccactttgcctttctctccacagggccgccaccatgaaacggacagccgacggaagcgagttcgagtcaccaaagaagaagcggaaagtctctgaggtggagttttcccacgagtactggatgagacatgccctgaccctggccaagagggcacgggatgagagggaggtgcctgtgggagccgtgctggtgctgaacaatagagtgatcggcgagggctggaacagagccatcggcctgcacgacccaacagcccatgccgaaattatggccctgagacagggcggcctggtcatgcagaactacagactgattgacgccaccctgtacgtgacattcgagccttgcgtgatgtgcgccggcgccatgatccactctaggatcggccgcgtggtgtttggcgtgaggaactcaaaaagaggcgccgcaggctccctgatgaacgtgctgaactaccccggcatgaatcaccgcgtcgaaattaccgagggaatcctggcagatgaatgtgccgccctgctgtgcgatttctatcggatgcctagacaggtgttcaatgctcagaagaaggcccagagctccatcaactccggaggatctagcggaggctcctctggctctgagacacctggcacaagcgagagcgcaacacctgaaagcagcgggggcagcagcggggggtcagcccgcatcctggcctttgccatcggcatcagcagcatcggatgggccttcagcgagaatgacgagctgaaggactgcggtgtgagaatctttacaaaggtcgagaaccccaagaccggcgaaagcctggcgctgccaagacggctggcccggtctgctcggaagagatacgcccggagaaaagccagactgaatcacctgaaacacctgatcgccaacgagttcaaactgaactacgaggactaccagagcttcgatgagagcttggctaaggcctacaaaggcagcctgatcagcccctacgagctgagattcagagctctgaatgagctcctgagcaagcaggacttcgctagagtgatcctgcacatcgccaagcgaagaggctacgacgacatcaagaactctgatgacaaggagaagggcgccattctgaaagccatcaagcagaacgaagagaaactggccaattaccagagcgtgggcgagtacctgtacaaggagtacttccagaagttcaaagaaaatagcaaagagttcaccaacgtgcggaacaagaaggagtcttatgaaagatgtatcgcccagagcttcctgaaagacgagctgaaactgatcttcaagaagcaaagagagtttggcttcagcttcagcaaaaaatttgaagaagaggtgctgtctgtcgccttctacaagagggctctgaaggacttcagccacctggtgggcaattgcagctttttcacagacgaaaagcgggcccctaagaacagccctctggccttcatgttcgtggctctgaccagaatcatcaacctgctgaacaacctgaaaaataccgagggcatcctctataccaaggacgatctgaacgccctgctgaatgaggtgctcaagaatggcaccctgacctacaagcaaacaaaaaaactgctgggcctgtctgacgactacgagtttaaaggcgagaagggcacctatttcatcgaatttaagaagtacaaggaattcatcaaggcactgggcgaacacaacctgtctcaggacgacctgaacgagatcgccaaggacatcaccctgatcaaggatgagatcaagctgaaaaaagctctggccaagtacgacctgaatcaaaaccagatcgacagcttaagcaagctggaatttaaggatcacctgaacatctcctttaaggccctgaagctggtgaccccactgatgctggaaggaaagaagtacgacgaagcatgcaacgagcttaacctgaaggttgctatcaacgaggataagaaggatttcctgcctgcctttaacgagacatactacaaggatgaggtgaccaaccccgtggtgctgagagctatcaaagagtacagaaaggtgctgaacgccctgctgaagaagtacggcaaggtccacaagatcaatattgagctggcccgggaggttggaaagaaccactctcagagagcaaagatcgagaaggagcaaaacgagaactacaaagcgaagaaggacgccgaactggagtgcgagaagcttggcctgaagatcaactctaagaatatcctgaaactcagacttttcaaagaacagaaggaattctgtgcctacagcggcgagaagatcaaaatttctgacctgcaggatgaaaagatgctggagatcgaccacatctacccttactccagaagcttcgacgacagctatatgaacaaagtgctggtgttcacaaagcagaaccaggagaagctgaatcagacccctttcgaggccttcggcaatgactccgccaagtggcagaaaatcgaggtgctggccaaaaacctgccaaccaagaaacagaagagaatcctcgacaagaactacaaggacaaggaacagaagaacttcaaggatcggaacctgaacgacacccggtacatcgccaggctggtgttaaattacaccaaggactacctggatttcctgcccctgagcgacgacgagaacaccaagctgaacgacacacagaagggcagcaaggtgcacgtggaagccaagagcggcatgctgaccagcgcactgcgccacacttggggcttcagcgctaaggaccggaacaaccacctgcatcacgccatcgatgccgtgatcatagcctacgccaacaactcaatcgtgaaagctttcagtgactttaagaaagaacaggagagcaactctgccgaactgtacgccaagaaaattagcgagctggactacaagaacaaacggaagttcttcgaacctttctcaggatttagacagaaggtgctggataagatcgatgaaatcttcgtgtccaagcccgagagaaagaagcctagcggagccctgcacaaggaaaccttcagaaaggaagaagagttctaccagtcttatgggggcaaagaaggcgtgctgaaggccctggaactcggcaagatcagaaaggtgaagggaaagattgtgaagaacggcgacatgttcagagtggacatcttcaagcacaagaagaccaacaagttctatgccgtgcctatctacacaatggatttcgccctgaaagtgctgcctaacaaggctgtcgccagatctaagaagggcgagatcaaggactggatcctgatggacgaaaactacgagttctgcttcagcctgtacaaggacagcctgatcctgatccaaacaaagaagatgcaggagcctgaattcgtgtactacaacgccttcacaagcagcaccgtgagcctgatcgtgtctaaacatgataacaagttcgaaaccctgtccaagaaccaaaagatcctgttcaagaacgccaacgagaaggaagtgatcgccaagggcatcggcattcagaatctgaaggtgttcgagaaatatatcgtgtccgctctgggagaggttacaaaggccgagtttcggcagagagaagattttaagaagtctggcggctcaaaaagaaccgccgacggcagcgaattcgagcccaagaagaagaggaaagtctaatagatctcgactgtgccttctagttgccagccatctgttgtttgcccctcccccgtgccttccttgaccctggaaggtgccactcccactgtcctttcctaataaaatgaggaaattgcatcgcattgtctgagtaggtgtcattctattctggggggtggggtggggcaggacagcaagggggaggattgggaagacaatagcaggcatgctggggatgcggtgggctctatggctcgagcggcccaaaaaaagcggttttaggggattgtaaccccgcagagtcccgcaaactctttattctagtcccttttcagggactagaacnnnnnnnnnnnnnnnnnnnnnnggtgtttcgtcctttccacaagatatataaagccaagaaatcgaaatactttcaagttacggtaagcatatgatagtccattttaaaacataattttaaaactgcaaactacccaagaaattattactttctacgtcacgtattttgtactaatatctttgtgtttacagtcaaattaattctaattatctctctaacagccttgtatcgtatatgcaaatatgaaggaatcatgggaaataggccctcaggaacccctagtgatggagttggccactccctctctgcgcgctcgctcgctcactgaggccgggcgaccaaaggtcgcccgacgcccgggctttgcccgggcggcctcagtgagcgagcgagcgcgcag

SEQ ID NO: 16 - DNA, 5004 bp, synthetic construct
  source 1..5004: mol_type = other DNA
ctgcgcgctcgctcgctcactgaggccgcccgggcaaagcccgggcgtcgggcgacctttggtcgcccggcctcagtgagcgagcgagcgcgcagagagggagtggccaactccatcactaggggttcctgagggccctgcgtatgagtgcaagtgggttttaggaccaggatgaggcggggtgggggtgcctacctgacgaccgaccccgacccactggacaagcacccaacccccattccccaaattgcgcatcccctatcagagagggggaggggaaacaggatgcggcgaggcgcgtgcgcactgccagcttcagcaccgcggacagtgccttcgcccccgcctggcggcgcgcgccaccgccgcctcagcactgaaggcgcgctgacgtcactcgccggtcccccgcaaactccccttcccggccaccttggtcgcgtccgcgccgccgccggcccagccggaccgcaccacgcgaggcgcgagataggggggcacgggcgcgaccatctgcgctgcggcgccggcgactcagcgctgcctcagtctgcggtgggcagcggaggagtcgtgtcgtgcctgagagcgcagtcgagaggccgccaccatgaaacggacagccgacggaagcgagttcgagtcaccaaagaagaagcggaaagtctctgaggtggagttttcccacgagtactggatgagacatgccctgaccctggccaagagggcacgggatgagagggaggtgcctgtgggagccgtgctggtgctgaacaatagagtgatcggcgagggctggaacagagccatcggcctgcacgacccaacagcccatgccgaaattatggccctgagacagggcggcctggtcatgcagaactacagactgattgacgccaccctgtacgtgacattcgagccttgcgtgatgtgcgccggcgccatgatccactctaggatcggccgcgtggtgtttggcgtgaggaactcaaaaagaggcgccgcaggctccctgatgaacgtgctgaactaccccggcatgaatcaccgcgtcgaaattaccgagggaatcctggcagatgaatgtgccgccctgctgtgcgatttctatcggatgcctagacaggtgttcaatgctcagaagaaggcccagagctccatcaactccggaggatctagcggaggctcctctggctctgagacacctggcacaagcgagagcgcaacacctgaaagcagcgggggcagcagcggggggtcagcccgcatcctggcctttgccatcggcatcagcagcatcggatgggccttcagcgagaatgacgagctgaaggactgcggtgtgagaatctttacaaaggtcgagaaccccaagaccggcgaaagcctggcgctgccaagacggctggcccggtctgctcggaagagatacgcccggagaaaagccagactgaatcacctgaaacacctgatcgccaacgagttcaaactgaactacgaggactaccagagcttcgatgagagcttggctaaggcctacaaaggcagcctgatcagcccctacgagctgagattcagagctctgaatgagctcctgagcaagcaggacttcgctagagtgatcctgcacatcgccaagcgaagaggctacgacgacatcaagaactctgatgacaaggagaagggcgccattctgaaagccatcaagcagaacgaagagaaactggccaattaccagagcgtgggcgagtacctgtacaaggagtacttccagaagttcaaagaaaatagcaaagagttcaccaacgtgcggaacaagaaggagtcttatgaaagatgtatcgcccagagcttcctgaaagacgagctgaaactgatcttcaagaagcaaagagagtttggcttcagcttcagcaaaaaatttgaagaagaggtgctgtctgtcgccttctacaagagggctctgaaggacttcagccacctggtgggcaattgcagctttttcacagacgaaaagcgggcccctaagaacagccctctggccttcatgttcgtggctctgaccagaatcatcaacctgctgaacaacctgaaaaataccgagggcatcctctataccaaggacgatctgaacgccctgctgaatgaggtgctcaagaatggcaccctgacctacaagcaaacaaaaaaactgctgggcctgtctgacgactacgagtttaaaggcgagaagggcacctatttcatcgaatttaagaagtacaaggaattcatcaaggcactgggcgaacacaacctgtctcaggacgacctgaacgagatcgccaaggacatcaccctgatcaaggatgagatcaagctgaaaaaagctctggccaagtacgacctgaatcaaaaccagatcgacagcttaagcaagctggaatttaaggatcacctgaacatctcctttaaggccctgaagctggtgaccccactgatgctggaaggaaagaagtacgacgaagcatgcaacgagcttaacctgaaggttgctatcaacgaggataagaaggatttcctgcctgcctttaacgagacatactacaaggatgaggtgaccaaccccgtggtgctgagagctatcaaagagtacagaaaggtgctgaacgccctgctgaagaagtacggcaaggtccacaagatcaatattgagctggcccgggaggttggaaagaaccactctcagagagcaaagatcgagaaggagcaaaacgagaactacaaagcgaagaaggacgccgaactggagtgcgagaagcttggcctgaagatcaactctaagaatatcctgaaactcagacttttcaaagaacagaaggaattctgtgcctacagcggcgagaagatcaaaatttctgacctgcaggatgaaaagatgctggagatcgaccacatctacccttactccagaagcttcgacgacagctatatgaacaaagtgctggtgttcacaaagcagaaccaggagaagctgaatcagacccctttcgaggccttcggcaatgactccgccaagtggcagaaaatcgaggtgctggccaaaaacctgccaaccaagaaacagaagagaatcctcgacaagaactacaaggacaaggaacagaagaacttcaaggatcggaacctgaacgacacccggtacatcgccaggctggtgttaaattacaccaaggactacctggatttcctgcccctgagcgacgacgagaacaccaagctgaacgacacacagaagggcagcaaggtgcacgtggaagccaagagcggcatgctgaccagcgcactgcgccacacttggggcttcagcgctaaggaccggaacaaccacctgcatcacgccatcgatgccgtgatcatagcctacgccaacaactcaatcgtgaaagctttcagtgactttaagaaagaacaggagagcaactctgccgaactgtacgccaagaaaattagcgagctggactacaagaacaaacggaagttcttcgaacctttctcaggatttagacagaaggtgctggataagatcgatgaaatcttcgtgtccaagcccgagagaaagaagcctagcggagccctgcacaaggaaaccttcagaaaggaagaagagttctaccagtcttatgggggcaaagaaggcgtgctgaaggccctggaactcggcaagatcagaaaggtgaagggaaagattgtgaagaacggcgacatgttcagagtggacatcttcaagcacaagaagaccaacaagttctatgccgtgcctatctacacaatggatttcgccctgaaagtgctgcctaacaaggctgtcgccagatctaagaagggcgagatcaaggactggatcctgatggacgaaaactacgagttctgcttcagcctgtacaaggacagcctgatcctgatccaaacaaagaagatgcaggagcctgaattcgtgtactacaacgccttcacaagcagcaccgtgagcctgatcgtgtctaaacatgataacaagttcgaaaccctgtccaagaaccaaaagatcctgttcaagaacgccaacgagaaggaagtgatcgccaagggcatcggcattcagaatctgaaggtgttcgagaaatatatcgtgtccgctctgggagaggttacaaaggccgagtttcggcagagagaagattttaagaagtctggcggctcaaaaagaaccgccgacggcagcgaattcgagcccaagaagaagaggaaagtctaatagatctcgactgtgccttctagttgccagccatctgttgtttgcccctcccccgtgccttccttgaccctggaaggtgccactcccactgtcctttcctaataaaatgaggaaattgcatcgcattgtctgagtaggtgtcattctattctggggggtggggtggggcaggacagcaagggggaggattgggaagacaatagcaggcatgctggggatgcggtgggctctatggctcgagcggcccaaaaaaagcggttttaggggattgtaaccccgcagagtcccgcaaactctttattctagtcccttttcagggactagaacnnnnnnnnnnnnnnnnnnnnnnggtgtttcgtcctttccacaagatatataaagccaagaaatcgaaatactttcaagttacggtaagcatatgatagtccattttaaaacataattttaaaactgcaaactacccaagaaattattactttctacgtcacgtattttgtactaatatctttgtgtttacagtcaaattaattctaattatctctctaacagccttgtatcgtatatgcaaatatgaaggaatcatgggaaataggccctcaggaacccctagtgatggagttggccactccctctctgcgcgctcgctcgctcactgaggccgggcgaccaaaggtcgcccgacgcccgggctttgcccgggcggcctcagtgagcgagcgagcgcgcag

SEQ ID NO: 17 - DNA, 5179 bp, synthetic construct
  source 1..5179: mol_type = other DNA
ctgcgcgctcgctcgctcactgaggccgcccgggcaaagcccgggcgtcgggcgacctttggtcgcccggcctcagtgagcgagcgagcgcgcagagagggagtggccaactccatcactaggggttcctaccggcgcgccgggggaggctgctggtgaatattaaccaaggtcaccccagttatcggaggagcaaacaggggctaagtccacacgcgtggtaccgtctgtctgcacatttcgtagagcgagtgttccgatactctaatctccctaggcaaggttcatatttgtgtaggttacttattctccttttgttgactaagtcaataatcagaatcagcaggtttggagtcagcttggcagggatcagcagcctgggttggaaggagggggtataaaagccccttcaccaggagaagccgtcacacagatccacaagctcctgggccgccaccatgaaacggacagccgacggaagcgagttcgagtcaccaaagaagaagcggaaagtcagtgatagcctcttgatgaatagacgcgaattcctgtatcagtttaaaaacgtgagatgggcaaaaggccgacgagagacatatctgtgctatgtcgttaagcgcagagattcagccaccagtttctctctcgacttcggctacctgcggaacaagaatggttgccatgttgagctcctgttcctgaggtatatcagcgactgggatttggacccagggcggtgctatagggtgacatggtttatttcctggtcaccttgttatgactgcgcgcggcatgttgccgattttctgagagggaaccctaacctgtctctgaggatcttcaccgcgcgactgtacttctgtgaggaccggaaagccgaacccgagggactgagacgcctccacagagcgggtgtgcagattgccataatgacctttaaggactacttctactgctggaacaccttcgtcgaaaatcacggccggactttcaaggcttgggaaggattgcatgaaaacagcgtcaggctttccaggcagcttcgccgcattcttctcccgtctggcggatctagcggaggatcctctggcagcgagacaccaggaacaagcgagtcagcaacaccagagagcagtggcggcagcagcggcgggtcagcccgcatcctggcctttgccatcggcatcagcagcatcggatgggccttcagcgagaatgacgagctgaaggactgcggtgtgagaatctttacaaaggtcgagaaccccaagaccggcgaaagcctggcgctgccaagacggctggcccggtctgctcggaagagatacgcccggagaaaagccagactgaatcacctgaaacacctgatcgccaacgagttcaaactgaactacgaggactaccagagcttcgatgagagcttggctaaggcctacaaaggcagcctgatcagcccctacgagctgagattcagagctctgaatgagctcctgagcaagcaggacttcgctagagtgatcctgcacatcgccaagcgaagaggctacgacgacatcaagaactctgatgacaaggagaagggcgccattctgaaagccatcaagcagaacgaagagaaactggccaattaccagagcgtgggcgagtacctgtacaaggagtacttccagaagttcaaagaaaatagcaaagagttcaccaacgtgcggaacaagaaggagtcttatgaaagatgtatcgcccagagcttcctgaaagacgagctgaaactgatcttcaagaagcaaagagagtttggcttcagcttcagcaaaaaatttgaagaagaggtgctgtctgtcgccttctacaagagggctctgaaggacttcagccacctggtgggcaattgcagctttttcacagacgaaaagcgggcccctaagaacagccctctggccttcatgttcgtggctctgaccagaatcatcaacctgctgaacaacctgaaaaataccgagggcatcctctataccaaggacgatctgaacgccctgctgaatgaggtgctcaagaatggcaccctgacctacaagcaaacaaaaaaactgctgggcctgtctgacgactacgagtttaaaggcgagaagggcacctatttcatcgaatttaagaagtacaaggaattcatcaaggcactgggcgaacacaacctgtctcaggacgacctgaacgagatcgccaaggacatcaccctgatcaaggatgagatcaagctgaaaaaagctctggccaagtacgacctgaatcaaaaccagatcgacagcttaagcaagctggaatttaaggatcacctgaacatctcctttaaggccctgaagctggtgaccccactgatgctggaaggaaagaagtacgacgaagcatgcaacgagcttaacctgaaggttgctatcaacgaggataagaaggatttcctgcctgcctttaacgagacatactacaaggatgaggtgaccaaccccgtggtgctgagagctatcaaagagtacagaaaggtgctgaacgccctgctgaagaagtacggcaaggtccacaagatcaatattgagctggcccgggaggttggaaagaaccactctcagagagcaaagatcgagaaggagcaaaacgagaactacaaagcgaagaaggacgccgaactggagtgcgagaagcttggcctgaagatcaactctaagaatatcctgaaactcagacttttcaaagaacagaaggaattctgtgcctacagcggcgagaagatcaaaatttctgacctgcaggatgaaaagatgctggagatcgaccacatctacccttactccagaagcttcgacgacagctatatgaacaaagtgctggtgttcacaaagcagaaccaggagaagctgaatcagacccctttcgaggccttcggcaatgactccgccaagtggcagaaaatcgaggtgctggccaaaaacctgccaaccaagaaacagaagagaatcctcgacaagaactacaaggacaaggaacagaagaacttcaaggatcggaacctgaacgacacccggtacatcgccaggctggtgttaaattacaccaaggactacctggatttcctgcccctgagcgacgacgagaacaccaagctgaacgacacacagaagggcagcaaggtgcacgtggaagccaagagcggcatgctgaccagcgcactgcgccacacttggggcttcagcgctaaggaccggaacaaccacctgcatcacgccatcgatgccgtgatcatagcctacgccaacaactcaatcgtgaaagctttcagtgactttaagaaagaacaggagagcaactctgccgaactgtacgccaagaaaattagcgagctggactacaagaacaaacggaagttcttcgaacctttctcaggatttagacagaaggtgctggataagatcgatgaaatcttcgtgtccaagcccgagagaaagaagcctagcggagccctgcacaaggaaaccttcagaaaggaagaagagttctaccagtcttatgggggcaaagaaggcgtgctgaaggccctggaactcggcaagatcagaaaggtgaagggaaagattgtgaagaacggcgacatgttcagagtggacatcttcaagcacaagaagaccaacaagttctatgccgtgcctatctacacaatggatttcgccctgaaagtgctgcctaacaaggctgtcgccagatctaagaagggcgagatcaaggactggatcctgatggacgaaaactacgagttctgcttcagcctgtacaaggacagcctgatcctgatccaaacaaagaagatgcaggagcctgaattcgtgtactacaacgccttcacaagcagcaccgtgagcctgatcgtgtctaaacatgataacaagttcgaaaccctgtccaagaaccaaaagatcctgttcaagaacgccaacgagaaggaagtgatcgccaagggcatcggcattcagaatctgaaggtgttcgagaaatatatcgtgtccgctctgggagaggttacaaaggccgagtttcggcagagagaagattttaagaagagcggcgggagcggcgggagcggggggagcactaatctgagcgacatcattgagaaggagactgggaaacagctggtcattcaggagtccatcctgatgctgcctgaggaggtggaggaagtgatcggcaacaagccagagtctgacatcctggtgcacaccgcctacgacgagtccacagatgagaatgtgatgctgctgacctctgacgcccccgagtataagccttgggccctggtcatccaggattctaacggcgagaataagatcaagatgctgtctggcggctcaaaaagaaccgccgacggcagcgaattcgagcccaagaagaagaggaaagtctaatagatctcgactgtgccttctagttgccagccatctgttgtttgcccctcccccgtgccttccttgaccctggaaggtgccactcccactgtcctttcctaataaaatgaggaaattgcatcgcattgtctgagtaggtgtcattctattctggggggtggggtggggcaggacagcaagggggaggattgggaagacaatagcaggcatgctggggatgcggtgggctctatggctcgagcggcccaaaaaaagcggttttaggggattgtaaccccgcagagtcccgcaaactctttattctagtcccttttcagggactagaacnnnnnnnnnnnnnnnnnnnnnnggtgtttcgtcctttccacaagatatataaagccaagaaatcgaaatactttcaagttacggtaagcatatgatagtccattttaaaacataattttaaaactgcaaactacccaagaaattattactttctacgtcacgtattttgtactaatatctttgtgtttacagtcaaattaattctaattatctctctaacagccttgtatcgtatatgcaaatatgaaggaatcatgggaaataggccctcaggaacccctagtgatggagttggccactccctctctgcgcgctcgctcgctcactgaggccgggcgaccaaaggtcgcccgacgcccgggctttgcccgggcggcctcagtgagcgagcgagcgcgcag

SEQ ID NO: 18 - DNA, 5131 bp, synthetic construct
  source 1..5131: mol_type = other DNA
ctgcgcgctcgctcgctcactgaggccgcccgggcaaagcccgggcgtcgggcgacctttggtcgcccggcctcagtgagcgagcgagcgcgcagagagggagtggccaactccatcactaggggttcctaccggcgcgccgggggaggctgctggtgaatattaaccaaggtcaccccagttatcggaggagcaaacaggggctaagtccacacgcgtggtaccgtctgtctgcacatttcgtagagcgagtgttccgatactctaatctccctaggcaaggttcatatttgtgtaggttacttattctccttttgttgactaagtcaataatcagaatcagcaggtttggagtcagcttggcagggatcagcagcctgggttggaaggagggggtataaaagccccttcaccaggagaagccgtcacacagatccacaagctcctgggccgccaccatgaaacggacagccgacggaagcgagttcgagtcaccaaagaagaagcggaaagtctctgaggtggagttttcccacgagtactggatgagacatgccctgaccctggccaagagggcacgggatgagaggaaggcccctgtgggagccgtgctggtgctgaacaatagagtgatcggcgagggctggaacagagccatcggcctgcacgacccaacagcccatgccgaaattatcgccctgagacagggcggcctggtcatgcagaactacagactgattgacgccaccctgtacgtgacattcgagccttgcgtgatgtgcgccggcgccatgatcaactctaggatcggccgcgtggtgtttggcgtgaggaactcaaaaagaggcgccgcaggctccctgatgaacgtgctgaactaccccggcatgaatcaccgcgtcgaaattaccgagggaatcctggcagatgaatgtgccgccctgctgtgcgatttctatcggatgcctagacaggtgttcaatgctcagaagaaggcccagagctccatcaactccggaggatctagcggaggctcctctggctctgagacacctggcacaagcgagagcgcaacacctgaaagcagcgggggcagcagcggggggtcagcccgcatcctggcctttgccatcggcatcagcagcatcggatgggccttcagcgagaatgacgagctgaaggactgcggtgtgagaatctttacaaaggtcgagaaccccaagaccggcgaaagcctggcgctgccaagacggctggcccggtctgctcggaagagatacgcccggagaaaagccagactgaatcacctgaaacacctgatcgccaacgagttcaaactgaactacgaggactaccagagcttcgatgagagcttggctaaggcctacaaaggcagcctgatcagcccctacgagctgagattcagagctctgaatgagctcctgagcaagcaggacttcgctagagtgatcctgcacatcgccaagcgaagaggctacgacgacatcaagaactctgatgacaaggagaagggcgccattctgaaagccatcaagcagaacgaagagaaactggccaattaccagagcgtgggcgagtacctgtacaaggagtacttccagaagttcaaagaaaatagcaaagagttcaccaacgtgcggaacaagaaggagtcttatgaaagatgtatcgcccagagcttcctgaaagacgagctgaaactgatcttcaagaagcaaagagagtttggcttcagcttcagcaaaaaatttgaagaagaggtgctgtctgtcgccttctacaagagggctctgaaggacttcagccacctggtgggcaattgcagctttttcacagacgaaaagcgggcccctaagaacagccctctggccttcatgttcgtggctctgaccagaatcatcaacctgctgaacaacctgaaaaataccgagggcatcctctataccaaggacgatctgaacgccctgctgaatgaggtgctcaagaatggcaccctgacctacaagcaaacaaaaaaactgctgggcctgtctgacgactacgagtttaaaggcgagaagggcacctatttcatcgaatttaagaagtacaaggaattcatcaaggcactgggcgaacacaacctgtctcaggacgacctgaacgagatcgccaaggacatcaccctgatcaaggatgagatcaagctgaaaaaagctctggccaagtacgacctgaatcaaaaccagatcgacagcttaagcaagctggaatttaaggatcacctgaacatctcctttaaggccctgaagctggtgaccccactgatgctggaaggaaagaagtacgacgaagcatgcaacgagcttaacctgaaggttgctatcaacgaggataagaaggatttcctgcctgcctttaacgagacatactacaaggatgaggtgaccaaccccgtggtgctgagagctatcaaagagtacagaaaggtgctgaacgccctgctgaagaagtacggcaaggtccacaagatcaatattgagctggcccgggaggttggaaagaaccactctcagagagcaaagatcgagaaggagcaaaacgagaactacaaagcgaagaaggacgccgaactggagtgcgagaagcttggcctgaagatcaactctaagaatatcctgaaactcagacttttcaaagaacagaaggaattctgtgcctacagcggcgagaagatcaaaatttctgacctgcaggatgaaaagatgctggagatcgaccacatctacccttactccagaagcttcgacgacagctatatgaacaaagtgctggtgttcacaaagcagaaccaggagaagctgaatcagacccctttcgaggccttcggcaatgactccgccaagtggcagaaaatcgaggtgctggccaaaaacctgccaaccaagaaacagaagagaatcctcgacaagaactacaaggacaaggaacagaagaacttcaaggatcggaacctgaacgacacccggtacatcgccaggctggtgttaaattacaccaaggactacctggatttcctgcccctgagcgacgacgagaacaccaagctgaacgacacacagaagggcagcaaggtgcacgtggaagccaagagcggcatgctgaccagcgcactgcgccacacttggggcttcagcgctaaggaccggaacaaccacctgcatcacgccatcgatgccgtgatcatagcctacgccaacaactcaatcgtgaaagctttcagtgactttaagaaagaacaggagagcaactctgccgaactgtacgccaagaaaattagcgagctggactacaagaacaaacggaagttcttcgaacctttctcaggatttagacagaaggtgctggataagatcgatgaaatcttcgtgtccaagcccgagagaaagaagcctagcggagccctgcacaaggaaaccttcagaaaggaagaagagttctaccagtcttatgggggcaaagaaggcgtgctgaaggccctggaactcggcaagatcagaaaggtgaagggaaagattgtgaagaacggcgacatgttcagagtggacatcttcaagcacaagaagaccaacaagttctatgccgtgcctatctacacaatggatttcgccctgaaagtgctgcctaacaaggctgtcgccagatctaagaagggcgagatcaaggactggatcctgatggacgaaaactacgagttctgcttcagcctgtacaaggacagcctgatcctgatccaaacaaagaagatgcaggagcctgaattcgtgtactacaacgccttcacaagcagcaccgtgagcctgatcgtgtctaaacatgataacaagttcgaaaccctgtccaagaaccaaaagatcctgttcaagaacgccaacgagaaggaagtgatcgccaagggcatcggcattcagaatctgaaggtgttcgagaaatatatcgtgtccgctctgggagaggttacaaaggccgagtttcggcagagagaagattttaagaagagcggcgggagcggcgggagcggggggagcactaatctgagcgacatcattgagaaggagactgggaaacagctggtcattcaggagtccatcctgatgctgcctgaggaggtggaggaagtgatcggcaacaagccagagtctgacatcctggtgcacaccgcctacgacgagtccacagatgagaatgtgatgctgctgacctctgacgcccccgagtataagccttgggccctggtcatccaggattctaacggcgagaataagatcaagatgctgtctggcggctcaaaaagaaccgccgacggcagcgaattcgagcccaagaagaagaggaaagtctaatagatctcgactgtgccttctagttgccagccatctgttgtttgcccctcccccgtgccttccttgaccctggaaggtgccactcccactgtcctttcctaataaaatgaggaaattgcatcgcattgtctgagtaggtgtcattctattctggggggtggggtggggcaggacagcaagggggaggattgggaagacaatagcaggcatgctggggatgcggtgggctctatggctcgagcggcccaaaaaaagcggttttaggggattgtaaccccgcagagtcccgcaaactctttattctagtcccttttcagggactagaacnnnnnnnnnnnnnnnnnnnnnnggtgtttcgtcctttccacaagatatataaagccaagaaatcgaaatactttcaagttacggtaagcatatgatagtccattttaaaacataattttaaaactgcaaactacccaagaaattattactttctacgtcacgtattttgtactaatatctttgtgtttacagtcaaattaattctaattatctctctaacagccttgtatcgtatatgcaaatatgaaggaatcatgggaaataggccctcaggaacccctagtgatggagttggccactccctctctgcgcgctcgctcgctcactgaggccgggcgaccaaaggtcgcccgacgcccgggctttgcccgggcggcctcagtgagcgagcgagcgcgcag

SEQ ID NO: 19 - DNA, 212 bp, synthetic construct
  source 1..212: mol_type = other DNA
gggcagagcgcacatcgcccacagtccccgagaagttggggggaggggtcggcaattgaaccggtgcctagagaaggtggcgcggggtaaactgggaaagtgatgtcgtgtactggctccgcctttttcccgagggtgggggagaaccgtatataagtgcagtagtcgccgtgaacgttctttttcgcaacgggtttgccgccagaacacag

SEQ ID NO: 20 - DNA, 99 bp, synthetic construct
  source 1..99: mol_type = other DNA
atatttgcatgtcgctatgtgttctgggaaatcaccataaacgtgaaatgtctttggatttgggaatcctcgaggttctgtatgagaccactctttccc

SEQ ID NO: 21 - DNA, 234 bp, synthetic construct
  source 1..234: mol_type = other DNA
atatttgcatgtcgctatgtgttctgggaaatcaccataaacgtgaaatgtctttggatttgggaatcctcgaggttctgtatgagaccactctttcccgggtaagtatcaaggttacaagacaggtttaaggagaccaatagaaactgggcttgtcgagacagagaagactcttgcgtttctgataggcacctattggtcttactgacatccactttgcctttctctccacag

SEQ ID NO: 22 - DNA, 355 bp, synthetic construct
  source 1..355: mol_type = other DNA
catcgggggagcagtcctccaaggactggccagtctccagatgcccgtgcacacaggaacactgccttatgcacgggagtcccagaagaaggggtgatttctttccccaccttagttacaccatcaagacccagccagggcatcccccctcctggcctgagggccagctccccatcctgaaaaacctgtctgctctccccacccctttgaggctatagggcccaaggggcaggttggactggattcccctccagcccctcccacccccaggacaaaatcagccaccccaggggcagggcctcacttgcctcaggaaccccagcctgccagcacctattccacctcccagcccagc

SEQ ID NO: 23 - DNA, 500 bp, synthetic construct
  source 1..500: mol_type = other DNA
catcctgagagatgagccaggacaaagaaccagtaatagctcctggagcagcacatctgttttgccaggattatcccttggatctcttaaaaccgagaccttgtaatctgaagactcaacttgggctgtacccttaaccttcagctctatgatgcaagtgagtccacaggaccggaggctttgagatgagcttttcagaagggaggagttggccgcttgctcccagagctccagcacctgcattcttctggctatgtcagaagccagatcatttccctcgttaaaaacaaaaacaaaaaaacaaacaaacaaaatgttagtctttgccctttatctgcctggcaaagcttttaattggcttgatctgtcattccgctagacataaaggggacaatccccggattaggaaggagctctccagctcgggtaaggagtctcaaggcaaggtaggcaagcaccaccggtccgcactctcgcccagcttttacgggaagaagaga

SEQ ID NO: 24 - DNA, 30 bp, synthetic construct
  source 1..30: mol_type = other DNA
gagtagaggcggccacgacctggtgnnnnn

SEQ ID NO: 25 - DNA, 30 bp, synthetic construct
  source 1..30: mol_type = other DNA
gttaggcagattccttatctggtgannnnn

SEQ ID NO: 26 - RNA, 103 nt, synthetic construct
  source 1..103: mol_type = other RNA
gagtagaggcggccacgacctggttttagtccctgaaaagggactaaaataaagagtttgcgggactctgcggggttacaatcccctaaaaccgcttttaaaa

SEQ ID NO: 27 - RNA, 103 nt, synthetic construct
  source 1..103: mol_type = other RNA
gttaggcagattccttatctgggttttagtccctgaaaagggactaaaataaagagtttgcgggactctgcggggttacaatcccctaaaaccgcttttaaaa

SEQ ID NO: 28 - DNA, 30 bp, synthetic construct
  source 1..30: mol_type = other DNA
ggttctcctattctcaggtccannnnnnnn

SEQ ID NO: 29 - DNA, 30 bp, synthetic construct
  source 1..30: mol_type = other DNA
ggttctcctattctcaggtccatcagacac

SEQ ID NO: 30 - DNA, 30 bp, synthetic construct
  source 1..30: mol_type = other DNA
gattctcctattctcaggtccatcagacat

SEQ ID NO: 31 - DNA, 30 bp, synthetic construct
  source 1..30: mol_type = other DNA
tgtcctcctggcatctggtctaccatcctc

SEQ ID NO: 32 - DNA, 30 bp, synthetic construct
  source 1..30: mol_type = other DNA
ggtgcacctaagatcagggcctgaacaaag

SEQ ID NO: 33 - DNA, 29 bp, synthetic construct
  source 1..29: mol_type = other DNA
acttctccatgagcaggtccatgaagtag

SEQ ID NO: 34 - DNA, 29 bp, synthetic construct
  source 1..29: mol_type = other DNA
acttctcctgtctcagggcccagagagca

SEQ ID NO: 35 - DNA, 30 bp, synthetic construct; identical to SEQ ID NO: 29
  source 1..30: mol_type = other DNA

SEQ ID NO: 36 - DNA, 30 bp, synthetic construct; identical to SEQ ID NO: 30
  source 1..30: mol_type = other DNA

SEQ ID NO: 37 - DNA, 30 bp, synthetic construct
  source 1..30: mol_type = other DNA
aattctcctattctcaggtccatcagccta

SEQ ID NO: 38 - DNA, 30 bp, synthetic construct
  source 1..30: mol_type = other DNA
tgctgttctctcctctgggccagatggagc

SEQ ID NO: 39 - DNA, 30 bp, synthetic construct
  source 1..30: mol_type = other DNA
ggccctccacatcccaggcctactcacctc

SEQ ID NO: 40 - DNA, 30 bp, synthetic construct
  source 1..30: mol_type = other DNA
ggtccttctgctctaggccccaggttcacc

SEQ ID NO: 41 - DNA, 30 bp, synthetic construct
  source 1..30: mol_type = other DNA
ggccaaactccagagataactannnnnnnn

SEQ ID NO: 42 - DNA, 30 bp, synthetic construct
  source 1..30: mol_type = other DNA
ggccaaactccagagataactaacccacac

SEQ ID NO: 43 - DNA, 30 bp, synthetic construct
  source 1..30: mol_type = other DNA
ggccaaactcccgagataactaacccactc

SEQ ID NO: 44 - DNA, 30 bp, synthetic construct
  source 1..30: mol_type = other DNA
gccccaggtccagagccaccttgtggagag

SEQ ID NO: 45 - DNA, 30 bp, synthetic construct
  source 1..30: mol_type = other DNA
ggccaaagcgcacagatggccatctggctg

SEQ ID NO: 46 - DNA, 30 bp, synthetic construct
  source 1..30: mol_type = other DNA
caccaaactcctctggtcactttcaaaaaa

SEQ ID NO: 47 - DNA, 30 bp, synthetic construct
  source 1..30: mol_type = other DNA
gaccaaaccctacaggttcctaggaatttc

SEQ ID NO: 48 - DNA, 30 bp, synthetic construct; identical to SEQ ID NO: 42
  source 1..30: mol_type = other DNA

SEQ ID NO: 49 - DNA, 30 bp, synthetic construct; identical to SEQ ID NO: 43
  source 1..30: mol_type = other DNA

SEQ ID NO: 50 - DNA, 30 bp, synthetic construct
  source 1..30: mol_type = other DNA
aaccaatctccagagataaccagagacaac

SEQ ID NO: 51 - DNA, 30 bp, synthetic construct
  source 1..30: mol_type = other DNA
agccagactccagagataatacggcacaag

SEQ ID NO: 52 - DNA, 30 bp, synthetic construct
  source 1..30: mol_type = other DNA
cacctgactccacagttagccaactgcagc

SEQ ID NO: 53 - DNA, 30 bp, synthetic construct
  source 1..30: mol_type = other DNA
gaaccaactcctgagataactaatccactc